European Patent Specification EP 4 120 999 B1, published September 10, 2025. Title: COMPOSITION, LIPID PARTICLE MANUFACTURING KIT, SUBSTANCE DELIVERY METHOD, AND DETECTION METHOD. Applicant: Shinshu University Kabushiki Kaisha Toshiba. The sequence listing filed with the application follows.

SEQUENCE LISTING (8 sequences)

SEQ ID NO: 1 - protein, 20 aa, artificial
  Nucleic acid condensing peptide
RQRQRYYRQRQRGGRRRRRR

SEQ ID NO: 2 - protein, 13 aa, artificial
  Nucleic acid condensing peptide
RQRQRGGRRRRRR

SEQ ID NO: 3 - protein, 21 aa, artificial
  nucleic acid condensing peptide
RRRRRRYYRQRQRGGRRRRRR

SEQ ID NO: 4 - protein, 39 aa, artificial
  Nucleic acid condensing peptide
GNQSSNFGPMKGGNFGGRSSGPYGGGGQYFAKPRNQGGY

SEQ ID NO: 5 - DNA, 516 bp, Oplophorus gracilirostrius
atggtcttcacactcgaagatttcgttggggactggcgacagacagccggctacaacctggaccaagtccttgaacagggaggtgtgtccagtttgtttcagaatctcggggtgtccgtaactccgatccaaaggattgtcctgagcggtgaaaatgggctgaagatcgacatccatgtcatcatcccgtatgaaggtctgagcggcgaccaaatgggccagatcgaaaaaatttttaaggtggtgtaccctgtggatgatcatcactttaaggtgatcctgcactatggcacactggtaatcgacggggttacgccgaacatgatcgactatttcggacggccgtatgaaggcatcgccgtgttcgacggcaaaaagatcactgtaacagggaccctgtggaacggcaacaaaattatcgacgagcgcctgatcaaccccgacggctccctgctgttccgagtaaccatcaacggagtgaccggctggcggctgtgcgaacgcattctggcgtaa

SEQ ID NO: 6 - RNA, 795 nt, artificial
  globin-leader + NanoLuc mRNA + poly(A)
gggagacaagcuugaauacaagcuacuuguucuuuuugcaccuguacggaaguguuacuucugcucuaaaagcugcggaauuguaccccuagcguuuaaacuuaagcuuggcaauccgguacuguugguaaagccaccauggucuucacacucgaagauuucguuggggacuggcgacagacagccggcuacaaccuggaccaaguccuugaacagggagguguguccaguuuguuucagaaucucgggguguccguaacuccgauccaaaggauuguccugagcggugaaaaugggcugaagaucgacauccaugucaucaucccguaugaaggucugagcggcgaccaaaugggccagaucgaaaaaauuuuuaaggugguguacccuguggaugaucaucacuuuaaggugauccugcacuauggcacacugguaaucgacgggguuacgccgaacaugaucgacuauuucggacggccguaugaaggcaucgccguguucgacggcaaaaagaucacuguaacagggacccuguggaacggcaacaaaauuaucgacgagcgccugaucaaccccgacggcucccugcuguuccgaguaaccaucaacggagugaccggcuggcggcugugcgaacgcauucuggcguaaggccgcgacucuagaacaacaacaauugcauucauuuuauguuucagguucagggggaggugugggagguuuuuucggauccucuagaggauccccgggcgagcucccaaaaaaaaaaaaaaaaaaaaaaaaaaaaaaccg

SEQ ID NO: 7 - DNA, 1209 bp, human
atgctcgagggagtgcaggtggaaaccatctccccaggagacgggcgcaccttccccaagcgcggccagacctgcgtggtgcactacaccgggatgcttgaagatggaaagaaagttgattcctcccgggacagaaacaagccctttaagtttatgctaggcaagcaggaggtgatccgaggctgggaagaaggggttgcccagatgagtgtgggtcagagagccaaactgactatatctccagattatgcctatggtgccactgggcacccaggcatcatcccaccacatgccactctcgtcttcgatgtggagcttctaaaactggaatctggcggtggatccggagtcgacggatttggtgatgtcggtgctcttgagagtttgaggggaaatgcagatttggcttacatcctgagcatggagccctgtggccactgcctcattatcaacaatgtgaacttctgccgtgagtccgggctccgcacccgcactggctccaacatcgactgtgagaagttgcggcgtcgcttctcctcgctgcatttcatggtggaggtgaagggcgacctgactgccaagaaaatggtgctggctttgctggagctggcgcagcaggaccacggtgctctggactgctgcgtggtggtcattctctctcacggctgtcaggccagccacctgcagttcccaggggctgtctacggcacagatggatgccctgtgtcggtcgagaagattgtgaacatcttcaatgggaccagctgccccagcctgggagggaagcccaagctctttttcatccaggcctgtggtggggagcagaaagaccatgggtttgaggtggcctccacttcccctgaagacgagtcccctggcagtaaccccgagccagatgccaccccgttccaggaaggtttgaggaccttcgaccagctggacgccatatctagtttgcccacacccagtgacatctttgtgtcctactctactttcccaggttttgtttcctggagggaccccaagagtggctcctggtacgttgagaccctggacgacatctttgagcagtgggctcactctgaagacctgcagtccctcctgcttagggtcgctaatgctgtttcggtgaaagggatttataaacagatgcctggttgctttaatttcctccggaaaaaacttttctttaaaacatcagctagctag

SEQ ID NO: 8 - RNA, 1383 nt, artificial
  globin-leader + iCaspase9 mRNA + poly(A)
gggagacaagcuugaauacaagcuacuuguucuuuuugcaccuguacggaaguguuacuucugcucuaaaagcugcggaauuguacccacuuaauacgacucacuauaggcuagacugccaugcucgagggagugcagguggaaaccaucuccccaggagacgggcgcaccuuccccaagcgcggccagaccugcguggugcacuacaccgggaugcuugaagauggaaagaaaguugauuccucccgggacagaaacaagcccuuuaaguuuaugcuaggcaagcaggaggugauccgaggcugggaagaagggguugcccagaugagugugggucagagagccaaacugacuauaucuccagauuaugccuauggugccacugggcacccaggcaucaucccaccacaugccacucucgucuucgauguggagcuucuaaaacuggaaucuggcgguggauccggagucgacggauuuggugaugucggugcucuugagaguuugaggggaaaugcagauuuggcuuacauccugagcauggagcccuguggccacugccucauuaucaacaaugugaacuucugccgugaguccgggcuccgcacccgcacuggcuccaacaucgacugugagaaguugcggcgucgcuucuccucgcugcauuucaugguggaggugaagggcgaccugacugccaagaaaauggugcuggcuuugcuggagcuggcgcagcaggaccacggugcucuggacugcugcgugguggucauucucucucacggcugucaggccagccaccugcaguucccaggggcugucuacggcacagauggaugcccugugucggucgagaagauugugaacaucuucaaugggaccagcugccccagccugggagggaagcccaagcucuuuuucauccaggccugugguggggagcagaaagaccauggguuugagguggccuccacuuccccugaagacgaguccccuggcaguaaccccgagccagaugccaccccguuccaggaagguuugaggaccuucgaccagcuggacgccauaucuaguuugcccacacccagugacaucuuuguguccuacucuacuuucccagguuuuguuuccuggagggaccccaagaguggcuccugguacguugagacccuggacgacaucuuugagcagugggcucacucugaagaccugcagucccuccugcuuagggucgcuaaugcuguuucggugaaagggauuuauaaacagaugccugguugcuuuaauuuccuccggaaaaaacuuuucuuuaaaacaucagcuagcuagaggauccccgggcgagcucccaaaaaaaaaaaaaaaaaaaaaaaaaaaaaaccg